European Patent Specification EP 3 849 305 B1, published December 13, 2023. Title: A GENETIC MOUSE MODEL OF AUTOIMMUNE ADVERSE EVENTS AND IMMUNE CHECKPOINT BLOCKADE THERAPY. Applicant: BOARD OF REGENTS, THE UNIVERSITY OF TEXAS SYSTEM. The sequence listing filed with the application follows.

SEQUENCE LISTING (6 sequences)

SEQ ID NO: 1 - DNA, 28 bp, Artificial sequence
  Synthetic primer
aaacaaccccaagctaactgcgacaagg

SEQ ID NO: 2 - DNA, 27 bp, Artificial sequence
  Synthetic primer
ccagaaccatgcccggattctgacttc

SEQ ID NO: 3 - DNA, 25 bp, Artificial sequence
  Synthetic primer
ccaagtgcccagcggggctgctaaa

SEQ ID NO: 4 - DNA, 21 bp, Artificial sequence
  Synthetic primer
cactatcccactgacccttca

SEQ ID NO: 5 - DNA, 20 bp, Artificial sequence
  Synthetic primer
agaaggtgagggacctccag

SEQ ID NO: 6 - DNA, 20 bp, Artificial sequence
  Synthetic primer
cacagggtaggcatgtagca